European Patent Specification EP 3 609 912 B1, published September 3, 2025. Title: METHODS TO PRODUCE PEPTIDES, POLYPEPTIDES OR CELLS FOR MODULATING IMMUNITY. Applicant: Imnate SA-arl. The sequence listing filed with the application follows.

SEQUENCE LISTING (21 sequences)

SEQ ID NO: 1 - protein, 13 aa, Homo sapiens
  MISC_FEATURE: epitope p53
KTYGGSYGFRLGF

SEQ ID NO: 2 - protein, 16 aa, Artificial Sequence
  CD8 Binding
KTYGGSYGFRLGFTQQ

SEQ ID NO: 3 - protein, 10 aa, Mycobacterium tuberculosis
  MISC_FEATURE: Epitope M. Tuberculosis
QQWNFAGIEA

SEQ ID NO: 4 - DNA, 8 bp, Artificial Sequence
  CpG ODN
acgttcgc

SEQ ID NO: 5 - protein, 9 aa, Homo sapiens
  MISC_FEATURE: Epitope MOG protein
FYWVSPGVL

SEQ ID NO: 6 - protein, 12 aa, Artificial Sequence
  SEQ 5 + motif CD4
FYWVSPGVLRYD

SEQ ID NO: 7 - protein, 11 aa, Homo sapiens
WCQVAQKFTGG

SEQ ID NO: 8 - protein, 14 aa, Artificial Sequence
  SEQ 10 (GAD65) + CD4 motif
WCQVAQKFTGGRYD

SEQ ID NO: 9 - protein, 14 aa, Artificial Sequence
  SEQ 8 modified
  LIPID (2)..(2): PALMITATE
WCQVAQKFTGGRYD

SEQ ID NO: 10 - protein, 8 aa, Dermatophagoides pteronyssinus
  MISC_FEATURE: DerP1
YWIVRNSW

SEQ ID NO: 11 - protein, 5 aa, Artificial Sequence
  CXHX motif
RCPHC

SEQ ID NO: 12 - protein, 13 aa, Artificial Sequence
  SEQs10+11
YWIVRNSWRCPHC

SEQ ID NO: 13 - protein, 11 aa, Haemophilus influenzae
FINAGYIFQHH

SEQ ID NO: 14 - protein, 14 aa, Artificial Sequence
  SEQ 14 + Cys and Cys
HCFINAGYIFQHHC

SEQ ID NO: 15 - protein, 524 aa, Homo sapiens
  MISC_FEATURE: Pompe disease
MYALFLLASLLGAALAGPVLGLKECTRGSAVWCQNVKTASDCGAVKHCLQTVWNKPTVKSLPCDICKDVVTAAGDMLKDNATEEEILVYLEKTCDWLPKPNMSASCKEIVDSYLPVILDIIKGEMSRPGEVCSALNLCESLQKHLAELNHQKQLESNKIPELDMTEVVAPFMANIPLLLYPQDGPRSKPGPKDNGDVCQDCIQMVTDIQTAVRTNSTFVQALVEHVKEECDRLGPGMADICKNYISQYSEIAIQMMMHMQPKEICALVGFCDEVKEMPMQTLVPAKVASKNVIPALELVEPIKKHEVPAKSDVYCEVCEFLVKEVTKLIDNNKTEKEILDAFDKMCSKLPKSLSEECQEVVDTYGSSILSILLEEVSPELVCSMLHLCSGTRLPALTVHVTQPKDGGFCEVCKKLVGYLDRNLEKNSTKQEILAALEKGCSFLPDPYQKQCDQFVAEYEPVLIEILVEVMDPSFVCLKIGACPSAHKPLLGTEKCIWGPSYWCQNTETAAQCNAVEHCKRHVWN

SEQ ID NO: 16 - protein, 524 aa, Artificial Sequence
  Mutated pompe
MYALFLLASLLGAALAGPVLGLKECTRGSAVWCQNVKTASDCGAVKHCLQTVWNKPTVKSLPCDICKDVVTAAGDMLKDNATEEEILVSLEKTCDALPKPNMSASCKEIVDSYLPVILDIIKGEMSRPGEVCSALNLCESLQKHLAELNHQKQLESNKIPELDMTEVVAPFMANIPLLLYPQDGPRSKPGPKDNGDVCQDCIQMVTDIQTAVRTNSTFVQALVEHVKEECDRLGPGMADICKNYISQYSEIAIQMMMHMQPKEICALVGFCDEVKEMPMQTLVPAKVASKNVIPALELVEPIKKHEVPAKSDVSCEVCEVLVKEVTKLIDNNKTEKEILDAFDKMCSKLPKSLSEECQEVVDTYGSSILSILLEEVSPELVCSMLHLCSGTRLPALTVHVTQPKDGGFCEVCKKLVGYLDRNLEKNSTKQEILAALEKGCSFLPDPYQKQCDQFVAEYEPVLIEILVEVMDPSFVCLKIGACPSAHKPLLGTEKCIWGPSYWCQNTETAAQCNAVEHCKRHVWN

SEQ ID NO: 17 - protein, 13 aa, Artificial Sequence
  AAV
FNGLDKGEPVNEA

SEQ ID NO: 18 - protein, 17 aa, Artificial Sequence
  SEQ 17 + Cys and Cys
HCFNGLDKGEPVNEACH

SEQ ID NO: 19 - protein, 12 aa, Artificial Sequence
  Celiac Disease
QLQPFPQPQLPY

SEQ ID NO: 20 - protein, 17 aa, Artificial Sequence
  SEQ I9 + CD4 motif
QLQPFPQPQLPYPQRYD

SEQ ID NO: 21 - protein, 14 aa, Artificial Sequence
  Flavivirus NS1 + CD8 motif
FIEVKSCHWSNTQQ